European Patent Specification EP 3 893 898 B1, published April 3, 2024. Title: METHOD OF TREATING AUTOIMMUNE AND INFLAMMATORY DISEASES USING B CELLS. Applicant: Versiti Blood Research Institute Foundation, Inc. Dittel, Bonnie N Khalil, Mohamed Ray, Avijit. The sequence listing filed with the application follows.

SEQUENCE LISTING (5 sequences)

SEQ ID NO: 1 - DNA, 23 bp, Artificial Sequence
  synthetic
tagtccttcctaccccaatttcc

SEQ ID NO: 2 - DNA, 21 bp, Artificial Sequence
  synthetic
ttggtccttagccactccttc

SEQ ID NO: 3 - DNA, 20 bp, Artificial Sequence
  synthetic
tgcagtatcccggagaaggg

SEQ ID NO: 4 - DNA, 22 bp, Artificial Sequence
  synthetic
ttctcatttccatagttctcac

SEQ ID NO: 5 - protein, 11 aa, Artificial Sequence
  synthetic
ASQKRPSQRSK